European Patent Application EP 4 122 959 A1, published January 25, 2023. Title: MULTISPECIFIC NANOBODIES CHIMERIC ANTIGEN RECEPTOR AND T-CELL ENGAGER, NUCLEIC ACID, EXPRESSING CELL THEREOF, AND PHARMACEUTICAL COMPOSITION FOR USE IN TREATMENT OF CANCER. Applicant: EVER SUPREME BIO TECHNOLOGY CO., LTD. Application EP 22186033.1, filed July 20, 2022. The sequence listing filed with the application follows.

SEQUENCE LISTING (30 sequences)

SEQ ID NO: 1 - protein, 124 aa, synthetic construct
EVQLVESGGGSVQAGGSLRLSCDASKYTYFRNCMGWFRQVPGAEREGVATIDSAGGTSYADFVKGRFTISRDNAKTALYLQMNSLKPEDTAMYYCFGGSWYKGSCIYEYNYWGQGTQVTVSSVD

SEQ ID NO: 2 - protein, 154 aa, synthetic construct
MKYLLPTAAAGLLLLAAQPAMAMGEVQLVESGGGSVQAGGSLRLSCDASKYTYFRNCMGWFRQVPGAEREGVATIDSAGGTSYADFVKGRFTISRDNAKTALYLQMNSLKPEDTAMYYCFGGSWYKGSCIYEYNYWGQGTQVTVSSLEHHHHHH

SEQ ID NO: 3 - DNA, 408 bp, synthetic construct
  source 1..408: mol_type = other DNA
atgggaagatctgagctcgaagttcagctggttgaaagtggtggcggtagcgtgcaggcaggtggtagcctgcgcctgagttgtgatgccagtaaatatacctacttccgtaattgtatgggttggttccgtcaggttccgggcgccgaacgcgaaggtgttgcaaccattgatagtgcaggcggcaccagttatgccgacttcgttaaaggtcgcttcaccattagccgtgataatgccaaaaccgcactgtatctgcagatgaatagtctgaaaccggaagataccgcaatgtattattgcttcggcggcagttggtataaaggtagctgtatctatgaatataactactggggtcagggtacccaggtgaccgttagcagcgtcgaccatcatcatcatcatcat

SEQ ID NO: 4 - DNA, 378 bp, synthetic construct
  source 1..378: mol_type = other DNA
atgggcgaagtgcagctggttgaaagcggtggtggcagcgttcaggcaggtggcagtctgcgcctgagttgcgatgccagtaaatatacctacttccgcaattgtatgggctggttccgtcaggtgccgggcgccgaacgcgaaggtgtggcaaccattgatagcgccggtggtaccagctatgccgacttcgtgaaaggtcgcttcaccattagccgcgataatgccaaaaccgcactgtatctgcagatgaatagcctgaaaccggaagataccgccatgtattattgcttcggcggcagctggtataaaggcagctgcatctatgaatataattattggggccagggcacccaggtgaccgttagtagtctcgag

SEQ ID NO: 5 - protein, 119 aa, synthetic construct
EVQLVESGGGLVQPGGSLRLSCVASGFTFSSIGMSWVRQAPGKGLEWVSGLNPVGSHTGYADSVKGRFTISRDNAKNTLHLQLNSLKTEDTAMYYCQRGYTCSGDLCERGQGTQVTVSS

SEQ ID NO: 6 - protein, 121 aa, synthetic construct
HVQLVESGGGLVQPGGSLRLSCAASGFTFSSKAMSWVRQAPGKGLDWVSTINSGGGNTYYSDSVKGRFTISRDNAKNTLYLQLNSLKTEDTAMYYCSRCSDIYCGGQYTYRGQGTLVTVSS

SEQ ID NO: 7 - DNA, 357 bp, synthetic construct
  source 1..357: mol_type = other DNA
gaggtgcagctggtggagtctgggggaggcttggtgcagcctggggggtctctgagactctcctgtgtagcctctggattcaccttcagtagcattggcatgagttgggtccgccaggctccagggaaggggctcgagtgggtctcaggtctgaatcctgttggtagtcacacaggctatgcagactccgtaaagggccgattcaccatctccagagacaacgccaagaatacgctgcatctgcagttgaacagcctgaaaactgaggacacggccatgtattactgtcaaagaggttatacttgtagcggtgatttgtgcgaaaggggtcaggggacccaggtcactgtctcctca

SEQ ID NO: 8 - DNA, 363 bp, synthetic construct
  source 1..363: mol_type = other DNA
catgtgcagctggtggagtctgggggaggcttggtgcagcctggggggtctctgagactctcctgtgcagcctctggattcaccttcagtagcaaggccatgagctgggtccgccaggctccagggaagggactcgactgggtctcaaccattaatagtggtggtggtaacacatactattcagactccgtgaagggccgattcaccatctccagagacaacgccaagaacacgctgtatctgcaattgaacagcctgaaaactgaggacacggccatgtattactgttcccgttgtagcgatatttactgcggagggcaatatacgtatcggggccaggggaccctggtcactgtctcctca

SEQ ID NO: 9 - protein, 128 aa, synthetic construct
HVQLVESGGGSVQAGGSLRLSCTVSGVIFKNEYMGWFRQAPGKEREGVAAASPGGTITYYGDSVKGRFTISRDNAKNTVYLQMNRLKPEDTAMYYCALDPSTTSWSIIRHGPSLWRYSGRGTQVTVSS

SEQ ID NO: 10 - DNA, 384 bp, synthetic construct
  source 1..384: mol_type = other DNA
catgtgcagctggtggagtctgggggaggctcggtgcaggctggggggtctctgagactctcctgtacagtgtctggagtcatctttaagaacgagtacatgggctggttccgccaggccccagggaaggagcgcgagggggtcgcagcagcttcgcctggtggaacgattacatactatggggactccgtgaagggccgattcaccatctcccgagacaatgccaagaacacggtgtatctgcaaatgaaccgcctgaaacctgaggacactgccatgtactactgtgcgttggatccctcgactacgtcatggtctatcatccgccacggtccatcgctttggcgttatagcggccgggggacccaggtcaccgtctcctca

SEQ ID NO: 11 - protein, 21 aa, synthetic construct
MALPVTALLLPLALLLHAARP

SEQ ID NO: 12 - DNA, 63 bp, synthetic construct
  source 1..63: mol_type = other DNA
atggccctccctgtcaccgccctgctgcttccgctggctcttctgctccacgccgctcggccc

SEQ ID NO: 13 - protein, 15 aa, synthetic construct
GGGGSGGGGSGGGGS

SEQ ID NO: 14 - DNA, 45 bp, synthetic construct
  source 1..45: mol_type = other DNA
ggaggcggaggttctggaggcggaggttctggaggcggaggttct

SEQ ID NO: 15 - protein, 20 aa, synthetic construct
MYRMQLLSCIALSLALVTNS

SEQ ID NO: 16 - DNA, 60 bp, synthetic construct
  source 1..60: mol_type = other DNA
atgtacaggatgcaactcctgtcttgcattgcactaagtcttgcacttgtcacaaacagt

SEQ ID NO: 17 - protein, 69 aa, synthetic construct
TTTPAPRPPTPAPTIASQPLSLRPEACRPAAGGAVHTRGLDFACDIYIWAPLAGTCGVLLLSLVITLYC

SEQ ID NO: 18 - DNA, 207 bp, synthetic construct
  source 1..207: mol_type = other DNA
accacgacgccagcgccgcgaccaccaacaccggcgcccaccatcgcgtcgcagcccctgtccctgcgcccagaggcgtgccggccagcggcggggggcgcagtgcacacgagggggctggacttcgcctgtgatatctacatttgggcccctctggctggtacttgcggggtcctgctgctttcactcgtgatcactctttactgt

SEQ ID NO: 19 - protein, 126 aa, synthetic construct
KVFLRCINYVFFPSLKPSSSIDEYFSEQPLKNLLLSTSEEQIERCFIIENISTIATVEETNQTPVQTTQEEDGCSCRFPEEEEGGCELDEDHKKYSSQTSQDSGNYSNEDESESKTSEELQLVLDS

SEQ ID NO: 20 - DNA, 378 bp, synthetic construct
  source 1..378: mol_type = other DNA
aaagtcttcttgagatgcatcaattatgtcttctttccatcacttaaaccttcttccagtatagatgagtatttctctgaacagccattgaagaatcttctgctttcaacttctgaggaacaaatcgaaagatgtttcataattgaaaatataagcacaattgctacagtagaagaaactaatcaaactccagtacaaactactcaagaggaagatggctgtagctgccgatttccagaagaagaagaaggaggatgtgaactggatgaagatcataaaaaatacagttcccaaactagccaagattcaggaaattattctaatgaagatgaaagcgaaagtaaaacaagtgaagaactacagctggtcttggactcc

SEQ ID NO: 21 - protein, 170 aa, synthetic construct
MAAGGPGAGSAAPVSSTSSLPLAALNMRVRRRLSLFLNVRTQVAADWTALAEEKKVAKKPTNKAPHPKMDFEYLEIRQLETQADPTGRLLDAWQGRPGASVGRLLELLTKLGCDDVLLELGPSIEEDCQKYILKQQQEEAEKPLQVAAVDSSVPRTAELAGITTLDDPLG

SEQ ID NO: 22 - DNA, 510 bp, synthetic construct
  source 1..510: mol_type = other DNA
atggctgcaggaggtcccggcgcggggtctgcggccccggtctcctccacatcctcccttcccctggctgctctcaacatgcgagtgcggcgccgcctgtctctgttcttgaacgtgcggacacaggtggcggccgactggaccgcgctggcggaggagaaaaaggtggccaagaagccaaccaataaggccccccaccccaagatggactttgagtacttggagatccggcaactggagacacaagcggaccccactggcaggctgctggacgcctggcagggacgccctggcgcctctgtaggccgactgctcgagctgcttaccaagctgggctgcgacgacgtgctgctggagctgggacccagcattgaggaggattgccaaaagtatatcttgaagcagcagcaggaggaggctgagaagcctttacaggtggccgctgtagacagcagtgtcccacggacagcagagctggcgggcatcaccacacttgatgaccccctgggg

SEQ ID NO: 23 - protein, 218 aa, synthetic construct
MAAGGPGAGSAAPVSSTSSLPLAALNMRVRRRLSLFLNVRTQVAADWTALAEEKVFLRCINYVFFPSLKPSSSIDEYFSEQPLKNLLLSTSEEQIERCFIIENISTIATVEETNQTMDFEYLEIRQLETQADPTGRLLDAWQGRPGASVGRLLELLTKLGCDDVLLELGPSIEEDCQKYILKQQQEEAEKPLQVAAVDSSVPRTAELAGITTLDDPLG

SEQ ID NO: 24 - DNA, 654 bp, synthetic construct
  source 1..654: mol_type = other DNA
atggctgcaggaggtcccggcgcggggtctgcggccccggtctcctccacatcctcccttcccctggctgctctcaacatgcgagtgcggcgccgcctgtctctgttcttgaacgtgcggacacaggtggcggccgactggaccgcgctggcggaggagaaagtcttcttgagatgcatcaattatgtcttctttccatcacttaaaccttcttccagtatagatgagtatttctctgaacagccattgaagaatcttctgctttcaacttctgaggaacaaatcgaaagatgtttcataattgaaaatataagcacaattgctacagtagaagaaactaatcaaactatggactttgagtacttggagatccggcaactggagacacaagcggaccccactggcaggctgctggacgcctggcagggacgccctggcgcctctgtaggccgactgctcgagctgcttaccaagctgggctgcgacgacgtgctgctggagctgggacccagcattgaggaggattgccaaaagtatatcttgaagcagcagcaggaggaggctgagaagcctttacaggtggccgctgtagacagcagtgtcccacggacagcagagctggcgggcatcaccacacttgatgaccccctgggg

SEQ ID NO: 25 - protein, 145 aa, synthetic construct
RVKFSRSADAPAYQQGQNQLYNELNLGRREEYDVLDKRRGRDPEMGGKPQRRKNPQEGLYNELQKDKMAEAYSEIGMKGERRRGKGHDGLYQGLSTATKDTYDALHMQYFLRKQRITETESPYQELQGQRSDVYSDLNTQALPPR

SEQ ID NO: 26 - DNA, 435 bp, synthetic construct
  source 1..435: mol_type = other DNA
agagtgaagttcagcaggagcgcagacgcccccgcgtaccagcagggccagaaccagctctataacgagctcaatctaggacgaagagaggagtacgatgttttggacaagagacgtggccgggaccctgagatggggggaaagccgcagagaaggaagaaccctcaggaaggcctgtacaatgaactgcagaaagataagatggcggaggcctacagtgagattgggatgaaaggcgagcgccggaggggcaaggggcacgatggcctttaccagggtctcagtacagccaccaaggacacctacgacgcccttcacatgcagtacttcctgcggaaacagcgtatcactgagaccgagtcgccttatcaggagctccagggtcagaggtcggatgtctacagcgacctcaacacacaggccctgccccctcgc

SEQ ID NO: 27 - protein, 19 aa, synthetic construct
ATNFSLLKQAGDVEENPGP

SEQ ID NO: 28 - DNA, 57 bp, synthetic construct
  source 1..57: mol_type = other DNA
gccacaaatttcagcctgctgaaacaggccggcgacgtggaagagaaccctggacct

SEQ ID NO: 29 - protein, 132 aa, synthetic construct
IISFFLALTSTALLFLLFFLTLRFSVVKRGRKKLLYIFKQPFMRKVFLRCINYVFFPSLKPSSSIDEYFSEQPLKNLLLSTSEEQIERCFIIENISTIATVEETNQTPVQTTQEEDGCSCRFPEEEEGGCEL

SEQ ID NO: 30 - DNA, 396 bp, synthetic construct
  source 1..396: mol_type = other DNA
atcatctccttctttcttgcgctgacgtcgactgcgttgctcttcctgctgttcttcctcacgctccgtttctctgttgttaaacggggcagaaagaaactcctgtatatattcaaacaaccatttatgagaaaagtcttcttgagatgcatcaattatgtcttctttccatcacttaaaccttcttccagtatagatgagtatttctctgaacagccattgaagaatcttctgctttcaacttctgaggaacaaatcgaaagatgtttcataattgaaaatataagcacaattgctacagtagaagaaactaatcaaactccagtacaaactactcaagaggaagatggctgtagctgccgatttccagaagaagaagaaggaggatgtgaactg